European Patent Specification EP 3 362 466 B1, published June 14, 2023. Title: AXMI554 DELTA-ENDOTOXIN GENE AND METHODS FOR ITS USE. Applicant: Bayer CropScience LP Bayer CropScience AG. The sequence listing filed with the application follows.

SEQUENCE LISTING (13 sequences)

SEQ ID NO: 1 - DNA, 846 bp, Pseudomonas putida
atgtgttgctacttactaaggaaggtaaaaatgagcacagttgatttggatgcaatcttcaagcgctacggtgattggtggtgcaagcaaaatggagggaagtgtgatcgcatgaatcctgttcagccgggctatgagcagcataggttgattgtgtccaacgaacatatcgagtactacggaaaccctaacaaggttgttgtgccacagatcgcgtctcagcaagttttggttaactctacttcagtggagcagtctcagtccgtgaggttttccaagactacgtcgagcacatttacgtggtctctgcaagaaggtatcaagcttgggatgtccgttacctataaggtgggtgtcgcccctatcatgtcggcggaaaccactattagtggcgaactgagcttctcgagcacgcaaacaaacacacagacagagaccaaaacttgggaggttgctcagcctgtcattgtccctgctaagactcaagttcaatccgttttggtaattgatgaaagtcgcgtcactcaaaagtttcacaataagtttacgttgagtggcagcgtttgtagtaatagcccaagtaagatcaatggtcactatttctggttccactcggtctcggatatatttaataagtttcctcagccgggctttaccgtgcgcagtgggcaggttttttacgagggcgatggtagctttgacggggtcgcggggattggaacccgactggaactcaccgaaagtccaattggtgatccatcaaaagtcctgaagacttatagtgtaattcctgtagtaccaggcgccggggtagcaaggctggctgatatggtcgatgagactgct

SEQ ID NO: 2 - DNA, 846 bp, Pseudomonas putida
atgtgctgctacctgctgcgtaaagtcaaaatgtcaacggtggacctggatgctatcttcaaacgctatggtgattggtggtgtaaacagaacggcggtaaatgcgatcgtatgaatccggtgcagccgggctatgaacaacatcgcctgattgttagtaacgaacacatcgaatattacggtaacccgaataaagtggttgtcccgcagattgccagccagcaagtcctggtgaattcaacctcggtggaacagagccagagcgtgcgtttttccaaaaccacgagctctaccttcacgtggtcactgcaggaaggcatcaaactgggcatgtcggttacctacaaagttggcgtcgctccgattatgtccgcggaaaccacgatctccggtgaactgtcatttagttccacccagacgaacacccaaacggaaaccaaaacgtgggaagtggcccagccggtgattgttccggcaaaaacccaggtccaatctgtcctggtgatcgatgaaagtcgcgtgacccagaaatttcataacaaattcacgctgagtggctccgtttgttcaaactcgccgagcaaaatcaacggtcattacttctggttccactctgtgagtgacatctttaataaattcccgcagccgggtttcaccgttcgtagcggtcaagtcttttacgaaggcgatggttctttcgacggcgttgctggcattggtacccgcctggaactgacggaatcgccgatcggtgatccgagcaaagtcctgaaaacctattctgtgattccggtggttccgggtgcgggtgttgcccgtctggcagatatggtcgacgaaacggca

SEQ ID NO: 3 - DNA, 816 bp, Pseudomonas putida
atgagcacggtggacctggacgctatcttcaaacgctacggcgactggtggtgtaaacaaaatggtggcaaatgtgaccgcatgaatccggtgcagccgggctatgaacaacatcgtctgattgttagtaacgaacacatcgaatattacggtaacccgaataaagtggttgtcccgcagattgccagccagcaagtcctggtgaattcaacctcggtggaacagagccagagcgtgcgcttttccaaaaccacgagctctaccttcacgtggtcactgcaggaaggcatcaaactgggcatgtcggttacctacaaagttggcgtcgctccgattatgtccgcggaaaccacgatctccggtgaactgtcatttagttccacccagacgaacacccaaacggaaaccaaaacgtgggaagtggcccagccggtgattgttccggcaaaaacccaggtccaatctgtcctggtgatcgatgaaagtcgtgtgacccagaaatttcataacaaattcacgctgagtggctccgtttgctcaaactcgccgagcaaaatcaacggtcattacttctggttccactctgtgagtgacatctttaataaattcccgcagccgggtttcaccgttcgtagcggtcaagtcttttacgaaggcgatggttctttcgacggcgttgctggcattggtacccgcctggaactgacggaatcgccgatcggtgatccgagcaaagtcctgaaaacctattctgtgattccggtggttccgggtgcgggtgttgcccgcctggcagatatggtcgacgaaacggca

SEQ ID NO: 4 - protein, 282 aa, Pseudomonas putida
MCCYLLRKVKMSTVDLDAIFKRYGDWWCKQNGGKCDRMNPVQPGYEQHRLIVSNEHIEYYGNPNKVVVPQIASQQVLVNSTSVEQSQSVRFSKTTSSTFTWSLQEGIKLGMSVTYKVGVAPIMSAETTISGELSFSSTQTNTQTETKTWEVAQPVIVPAKTQVQSVLVIDESRVTQKFHNKFTLSGSVCSNSPSKINGHYFWFHSVSDIFNKFPQPGFTVRSGQVFYEGDGSFDGVAGIGTRLELTESPIGDPSKVLKTYSVIPVVPGAGVARLADMVDETA

SEQ ID NO: 5 - protein, 272 aa, Pseudomonas putida
MSTVDLDAIFKRYGDWWCKQNGGKCDRMNPVQPGYEQHRLIVSNEHIEYYGNPNKVVVPQIASQQVLVNSTSVEQSQSVRFSKTTSSTFTWSLQEGIKLGMSVTYKVGVAPIMSAETTISGELSFSSTQTNTQTETKTWEVAQPVIVPAKTQVQSVLVIDESRVTQKFHNKFTLSGSVCSNSPSKINGHYFWFHSVSDIFNKFPQPGFTVRSGQVFYEGDGSFDGVAGIGTRLELTESPIGDPSKVLKTYSVIPVVPGAGVARLADMVDETA

SEQ ID NO: 6 - protein, 245 aa, Pseudomonas putida
MNPVQPGYEQHRLIVSNEHIEYYGNPNKVVVPQIASQQVLVNSTSVEQSQSVRFSKTTSSTFTWSLQEGIKLGMSVTYKVGVAPIMSAETTISGELSFSSTQTNTQTETKTWEVAQPVIVPAKTQVQSVLVIDESRVTQKFHNKFTLSGSVCSNSPSKINGHYFWFHSVSDIFNKFPQPGFTVRSGQVFYEGDGSFDGVAGIGTRLELTESPIGDPSKVLKTYSVIPVVPGAGVARLADMVDETA

SEQ ID NO: 7 - protein, 172 aa, Pseudomonas putida
MSVTYKVGVAPIMSAETTISGELSFSSTQTNTQTETKTWEVAQPVIVPAKTQVQSVLVIDESRVTQKFHNKFTLSGSVCSNSPSKINGHYFWFHSVSDIFNKFPQPGFTVRSGQVFYEGDGSFDGVAGIGTRLELTESPIGDPSKVLKTYSVIPVVPGAGVARLADMVDETA

SEQ ID NO: 8 - protein, 160 aa, Pseudomonas putida
MSAETTISGELSFSSTQTNTQTETKTWEVAQPVIVPAKTQVQSVLVIDESRVTQKFHNKFTLSGSVCSNSPSKINGHYFWFHSVSDIFNKFPQPGFTVRSGQVFYEGDGSFDGVAGIGTRLELTESPIGDPSKVLKTYSVIPVVPGAGVARLADMVDETA

SEQ ID NO: 9 - protein, 282 aa, Pseudomonas putida; identical to SEQ ID NO: 4

SEQ ID NO: 10 - protein, 282 aa, Pseudomonas putida; identical to SEQ ID NO: 4

SEQ ID NO: 11 - protein, 282 aa, Pseudomonas putida; identical to SEQ ID NO: 4

SEQ ID NO: 12 - protein, 4 aa, Artificial sequence
  endoplasmic reticulum targeting peptide
KDEL

SEQ ID NO: 13 - DNA, 819 bp, Artificial sequence
  synthetic gene encoding Axmi554
atgagcactgtggatttggatgccatcttcaagagatatggagattggtggtgcaagcagaatggaggaaaatgtgacaggatgaaccctgtgcaacctggatatgagcagcacaggttgattgtttccaatgagcacattgaatattatggaaatccaaacaaggtggtggttcctcagattgcttctcagcaagtgctggtcaactcaacttctgtggagcaaagccaaagtgtgaggttctccaagacaacaagctcaaccttcacttggagcttgcaagaaggaatcaagctggggatgagtgtcacctacaaggttggagttgctccaatcatgagtgctgaaacaacaatttctggagagttgagcttctcttcaacccaaaccaacacccaaacagaaaccaagacatgggaagtggctcaaccagtgattgttcctgccaagacccaagtgcaaagtgtgctggtgattgatgaaagcagagtgacccagaagttccacaacaagttcaccctctctggaagtgtttgcagcaattctccaagcaagatcaatggccattacttctggttccattctgtttcagacatcttcaacaagtttcctcaacctggcttcactgtgaggagtggccaagttttttatgaaggagatggaagttttgatggagttgctggaattggaacaaggttggagctgacagaaagcccaattggagatccttcaaaggtgctgaagacatattctgtgattccagtggttcctggtgctggagtggcaaggcttgctgacatggtggatgaaactgcttga